European Patent Application EP 4 461 305 A2, published November 13, 2024. Title: 녹차 펩타이드 조성물을 포함하는 혈당 강하용 조성물. Applicant: (주)아모레퍼시픽. The sequence listing filed with the application follows.

SEQUENCE LISTING (7 sequences)

SEQ ID NO: 1 - protein, 10 aa, unidentified
AYKRRKGKFA

SEQ ID NO: 2 - protein, 17 aa, unidentified
FFFFFFFFFFFFFFFYL

SEQ ID NO: 3 - protein, 21 aa, unidentified
ISKIWNSEVPETEVKNEAESP

SEQ ID NO: 4 - protein, 11 aa, unidentified
PFFCEKMMETN

SEQ ID NO: 5 - protein, 11 aa, unidentified
RFLHERMAYYH

SEQ ID NO: 6 - protein, 29 aa, unidentified
RNLNRLQRLLSMKQEYSPRNHLGSRWREY

SEQ ID NO: 7 - protein, 26 aa, unidentified
TTSSRKKEKPRRFWNNHEEVFLITTK